European Patent Specification EP 3 943 599 B1, published October 1, 2025. Title: AMINOACYL-TRNA SYNTHETASE FOR EFFICIENTLY INTRODUCING LYSINE             DERIVATIVE IN PROTEIN. Applicant: NINGBO KUNPENG BIOTECH CO., LTD. The sequence listing filed with the application follows.

SEQUENCE LISTING (13 sequences)

SEQ ID NO: 1 - protein, 454 aa, Methanosarcina mazei
MDKKPLNTLISATGLWMSRTGTIHKIKHHEVSRSKIYIEMACGDHLVVNNSRSSRTARALRHHKYRKTCKRCRVSDEDLNKFLTKANEDQTSVKVKVVSAPTRTKKAMPKSVARAPKPLENTEAAQAQPSGSKFSPAIPVSTQESVSVPASVSTSISSISTGATASALVKGNTNPITSMSAPVQASAPALTKSQTDRLEVLLNPKDEISLNSGKPFRELESELLSRRKKDLQQIYAEERENYLGKLEREITRFFVDRGFLEIKSPILIPLEYIERMGIDNDTELSKQIFRVDKNFCLRPMLAPNLYNYLRKLDRALPDPIKIFEIGPCYRKESDGKEHLEEFTMLNFCQMGSGCTRENLESIITDFLNHLGIDFKIVGDSCMVYGDTLDVMHGDLELSSAVVGPIPLDREWGIDKPWIGAGFGLERLLKVKHDFKNIKRAARSESYYNGISTNL

SEQ ID NO: 2 - protein, 454 aa, Methanosarcina mazei
MDKKPLNTLISATGLWMSRTGTIHKIKHHEVSRSKIYIEMACGDHLVVNNSRSSRTARALRHHKYRKTCKRCRVSDEDLNKFLTKANEDQTSVKVKVVSAPTRTKKAMPKSVARAPKPLENTEAAQAQPSGSKFSPAIPVSTQESVSVPASVSTSISSISTGATASALVKGNTNPITSMSAPVQASAPALTKSQTDRLEVLLNPKDEISLNSGKPFRELESELLSRRKKDLQQIYAEERENYLGKLEREITRFFVDRGFLEIKSPILIPLEYIERMGIDNDTELSKQIFRVDKNFCLRPMLAPNLYNYLRKLDRALPDPIKIFEIGPCYRKESDGKEHLEEFTMLNFCQMGSGCTRENLESIITDFLNHLGIDFKIVGDSCMVYGDTLDVMHGDLELSSAVVGPIPLDREWGIDKPWIGAGFGLERLLKVKHDFKNIKRAARSGSYYNGISTNL

SEQ ID NO: 3 - protein, 454 aa, artificial sequence
  mutant lysyl-tRNA synthetase
MDKKPLNTLISATGLWMSHTGTIHKVKHREVSRSKIYIEMACGDHLVVNNSRSSRTARALRHHKYRKTCKRCRVSDEDLNKFLTKANEDQTSVKVKVVSAPTRTKKAMPKSVARAPKPLENTEAAQAQPSGSKFSPAIPVSTQESVSVPASVSTSISSISTGATASALVKGNTNPITSMSAPVQASAPALTKSQTDRLEVLLNPKDEISLNSGKPFRELESELLSRRKKDLQQIYAEERENYLGKLEREITRFFVDRGFLEIKSPILIPLEYIERMGIDNDTELSKQIFRVDKNFCLRPMLAPNLYNYLRKLDRALPDPIKIFEIGPCYRKESDGKEHLEEFTMLNFCQMGSGCTRENLESIITDFLNHLGIDFKIVGDSCMVYGDTLDVMHGDLELSSAVVGPIPLDREWGIDKPWIGAGFGLERLLKVKHDFKNIKRAARSESYYNGISTNL

SEQ ID NO: 4 - protein, 454 aa, artificial sequence
  mutant lysyl-tRNA synthetase
MDKKPLNTLISATGLWMSHTGTIHKIKHREVSRSKIYIEMACGDHLVVNNSRSSRTARALRHHKYRKTCKRCRVSDEDLNKFLTKANEDQTSVKVKVVSAPTRTKKAMPKSVARAPKPLENSEAAQAQPSGSKFSPAIPVSTQESVSVPASVSTSISSISTGATASALVKGNTNPITSMSAPVQASAPALTKSQTDRLEVLLNPKDEISLNSGKPFRELESELLSRRKKDLQQIYAEERENYLGKLEREITRFFVDRGFLEIKSPILIPLEYIERMGIDNDTELSKQIFRVDKNFCLRPMLAPNLYNYLRKLDRALPDPIKIFEIGPCYRKESDGKEHLEEFTMLNFCQMGSGCTRENLESIITDFLNHLGIDFKIVGDSCMVFGDTLDVMHGDLELSSAVVGPIPLDREWGIDKPWIGAGFGLERLLKVKHDFKNIKRAARSESYYNGISTNL

SEQ ID NO: 5 - protein, 454 aa, artificial sequence
  mutant lysyl-tRNA synthetase
MDKKPLNTLISATGLWMSHTGTIHKIKHREVSRSKIYIEMACGDHLVVNNSRSSRTARALRHHKYRKTCKRCRVSDEDLNKFLTKANEDQTSVKVKVVSAPTRTKKAMPKSVARAPKPLENTEAAQAQPSGSKFSPAIPVSTQESVSVPASVSTSISSISTGATASALVKGNTNPITSMSAPVQASAPALTKSQTDRLEVLLNPKDEISLNSGKPFRELESELLSRRKKDLQQIYAEERENYLGKLEREITRFFVDRGFLEIKSPILIPLEYIERMGIDNDTELSKQIFRVDKNFCLRPMLAPNLYNYARKLDRALPDPIKIFEIGPCYRKESDGKEHLEEFTMLNFSQMGSGCTRENLESIITDFLNHLGIDFKIVGDSCMVYGDTLDVMHGDLELSSAVVGPIPLDREWGIDKPWIGAGFGLERLLKVKHDFKNIKRAARSESYYNGISTNL

SEQ ID NO: 6 - protein, 454 aa, artificial sequence
  mutant lysyl-tRNA synthetase
MDKKPLNTLISATGLWMSHTGTIHKIKHREVSRSKIYIEMACGDHLVVNNSRSSRTARALRHHKYRKTCKRCRVSDEDLNKFLTKANEDQTSVKVKVVSAPTRTKKAMPKSVARAPKPLENTEAAQAQPSGSKFSPAIPVSTQESVSVPASVSTSISSISTGATASALVKGNTNPITSMSAPVQASAPALTKSQTDRLEVLLNPKDEISLNSGKPFRELESELLSRRKKDLQQIYAEERENYLGKLEREITRFFVDRGFLEIKSPILIPLEYIERMGIDNDTELSKQIFRVDKNFCLRPMLAPNLYNYLRKLDRALPDPIKIFEIGPCYRKESDGKEHLEEFTMLNFCQMGSGCTRENLESIITDFLNHLGIDFKIVGDSCMVYGDTLDVMHGDLELSSAVVGPIPLDREWGIDKPWIGAGFGLERLLKVKHDFKNIKRAARSESYYNGISTNL

SEQ ID NO: 7 - protein, 454 aa, artificial sequence
  mutant lysyl-tRNA synthetase
MDKKPLNTLISATGLWMSHTGTIHKIKHHEVSRSKIYIEMACGDHLVVNNSRSSRTARALRHHKYRKTCKRCRVSDEDLNKFLTKANEDQTSVKVKVVSAPTRTKKAMPKSVARAPKPLENTEAAQAQPSGSKFSPAIPVSTQESVSVPASVSTSISSISTGATASALVKGNTNPITSMSAPVQASAPALTKSQTDRLEVLLNPKDEISLNSGKPFRELESELLSRRKKDLQQIYAEERENYLGKLEREITRFFVDRGFLEIKSPILIPLEYIERMGIDNDTELSKQIFRVDKNFCLRPMLAPNLYNYLRKLDRALPDPIKIFEIGPCYRKESDGKEHLEEFTMLNFCQMGSGCTRENLESIITDFLNHLGIDFKIVGDSCMVYGDTLDVMHGDLELSSAVVGPIPLDREWGIDKPWIGAGFGLERLLKVKHDFKNIKRAARSESYYNGISTNL

SEQ ID NO: 8 - protein, 454 aa, artificial sequence
  mutant lysyl-tRNA synthetase
MDKKPLNTLISATGLWMSRTGTIHKIKHREVSRSKIYIEMACGDHLVVNNSRSSRTARALRHHKYRKTCKRCRVSDEDLNKFLTKANEDQTSVKVKVVSAPTRTKKAMPKSVARAPKPLENTEAAQAQPSGSKFSPAIPVSTQESVSVPASVSTSISSISTGATASALVKGNTNPITSMSAPVQASAPALTKSQTDRLEVLLNPKDEISLNSGKPFRELESELLSRRKKDLQQIYAEERENYLGKLEREITRFFVDRGFLEIKSPILIPLEYIERMGIDNDTELSKQIFRVDKNFCLRPMLAPNLYNYLRKLDRALPDPIKIFEIGPCYRKESDGKEHLEEFTMLNFCQMGSGCTRENLESIITDFLNHLGIDFKIVGDSCMVYGDTLDVMHGDLELSSAVVGPIPLDREWGIDKPWIGAGFGLERLLKVKHDFKNIKRAARSESYYNGISTNL

SEQ ID NO: 9 - DNA, 72 bp, artificial sequence
  the encoding nucleic acid sequence of the orthogonal tRNA
ggaaacctgatcatgtagatcgaatggactctaaatccgttcagccgggttagattcccggggtttccgcca

SEQ ID NO: 10 - DNA, 20 bp, artificial sequence
  primer
ataccggcaccatccacaag

SEQ ID NO: 11 - DNA, 20 bp, artificial sequence
  primer
ggctcatccacagaccagtt

SEQ ID NO: 12 - DNA, 20 bp, artificial sequence
  primer
gcgaggtttcccgtagcaaa

SEQ ID NO: 13 - DNA, 22 bp, artificial sequence
  primer
ggtgtttgatcttgtggatggt